European Patent Application EP 4 555 975 A2, published May 21, 2025. Title: Beschichtetes Haar und dessen Verwendung. Applicant: Strauch, Georg. The sequence listing filed with the application follows.

SEQUENCE LISTING (13 sequences)

SEQ ID NO: 1 - skipped

SEQ ID NO: 2 - protein, 5 aa, synthetic construct
  REGION 1..5: note; note (original language) = Wiederholungssequenz aus Seidenprotein
  MOD_RES 5: note; note (original language) = jedes X kann unabhaengig voneinander jede beliebige natuerliche Aminosaeure sein
GVPGX

SEQ ID NO: 3-6 - skipped (4 entries)

SEQ ID NO: 7 - protein, 5263 aa, Bombyx mori
MRVKTFVILCCALQYVAYTNANINDFDEDYFGSDVTVQSSNTTDEIIRDASGAVIEEQITTKKMQRKNKNHGILGKNEKMIKTFVITTDSDGNESIVEEDVLMKTLSDGTVAQSYVAADAGAYSQSGPYVSNSGYSTHQGYTSDFSTSAAVGAGAGAGAAAGSGAGAGAGYGAASGAGAGAGAGAGAGYGTGAGAGAGAGYGAGAGAGAGAGYGAGAGAGAGAGYGAGAGAGAGAGYGAGAGAGAGAGYGAGAGAGAGAGYGAASGAGAGAGYGQGVGSGAASGAGAGAGAGSAAGSGAGAGAGTGAGAGYGAGAGAGAGAGYGAASGTGAGYGAGAGAGYGGASGAGAGAGAGAGAGAGAGYGTGAGYGAGAGAGAGAGAGAGYGAGAGAGYGAGYGVGAGAGYGAGYGAGAGSGAASGAGSGAGAGSGAGAGSGAGAGSGAGAGSGAGAGSGAGAGSGAGAGSGAGAGSGTGAGSGAGAGYGAGAGAGYGAGAGSGAASGAGAGSGAGAGSGAGAGSGAGAGSGAGAGSGAGAGYGAGAGAGYGAGAGAGYGAGAGVGYGAGAGSGAASGAGAGSGAGAGSGAGAGSGAGAGSGAGAGSGAGAGSGAGAGSGAGAGSGAGAGSGAGVGYGAGVGAGYGAGYGAGAGAGYGAGAGSGAASGAGAGAGAGAGTGSSGFGPYVANGGYSRSDGYEYAWSSDFGTGSGAGAGSGAGAGSGAGAGSGAGAGSGAGAGSGAGAGYGAGVGVGYGAGYGAGAGAGYGAGAGSGAASGAGAGSGAGAGSGAGAGSGAGAGSGAGAGSGAGAGSGAGAGSGAGAGSGAGAGSGAGAGSGAGVGSGAGAGSGAGAGVGYGAGAGVGYGAGAGSGAASGAGAGSGAGAGSGAGAGSGAGAGSGAGAGSGAGAGSGAGAGSGAGAGSGAGAGSGAGVGYGAGVGAGYGAGYGAGAGAGYGAGAGSGAASGAGAGSGAGAGSGAGAGSGAGAGSGAGAGSGAGAGSGAGAGSGAGAGSGAGAGSGAGAGSGAGAGSGAGAGYGAGAGAGYGAGYGAGAGAGYGAGAGSGAASGAGSGAGAGSGAGAGAGSGAGAGSGAGAGSGAGAGSGAGAGSGAGAGSGAGAGYGAGVGAGYGAGYGAGAGAGYGAGAGSGAASGAGAGSGAGAGSGAGAGSGAGAGSGAGAGSGAGAGSGAGAGSGAGVGYGAGYGAGAGAGYGAGAGSGAASGAGAGAGAGAGTGSSGFGPYVAHGGYSGYEYAWSSESDFGTGSGAGAGSGAGAGSGAGAGSGAGAGSGAGYGAGVGAGYGAGYGAGAGAGYGAGAGSGAGSGAGAGSGAGAGSGAGAGSGAGAGSGAGAGSGAGAGSGAGAGSGAGAGSGAGAGYGAGYGAGAGAGYGAGAGSGAGSGAGAGSGAGAGSGAGAGSGAGAGSGAGAGSGAGAGSGAGAGSGAGAGYGAGVGAGYGAGYGAGAGAGYGAGAGSGAGSGAGAGSGAGAGSGAGAGSGAGVGSGAGAGSGAGAGSGAGAGSGAGAGYGAGYGAGAGAGYGAGAGSGAGSGAGAGSGAGAGSGAGAGSGAGAGSGAGAGSGAGAGSGAGAGSGAGVGYGAGVGAGYGAGYGAGAGAGYGAGAGSGAASGAGAGAGAGAGTGSSGFGPYVANGGYSGYEYAWSSESDFGTGSGAGAGSGAGAGSGAGAGSGAGAGSGAGAGYGAGYGAGAGAGYGAGAGSGAGSGAGAGSGAGAGSGAGAGSGAGAGSGAGAGSGAGAGSGAGAGSGAGSGSGAGAGSGAGAGSGAGAGYGAGVGAGYGVGYGAGAGAGYGAGAGSGAASGAGAGAGAGAGTGSSGFGPYVAHGGYSGYEYAWSSESDFGTGSGAGAGSGAGAGSGAGAGSGAGAGSGAGAGSGAGAGSGAGAGYGAGVGAGYGAAYGAGAGAGYGAGAGSGAASGAGAGSGAGAGSGAGAGSGAGAGSGAGAGSGAGAGSGAGAGSGAGAGSGAGAGSGAGAGSGAGAGYGAGAGAGYGAGAGSGAGSGAGAGSGAGAGSGAGAGSGAGAGSGAGAGSGAGSGSGAGAGSGAGAGSGAGAGYGAGVGAGYGAGYGAGAGAGYGAGAGSGAGSGAGAGSGAGAGYGAGAGAGYGAGYGAGAGAGYGAGAGTGAGSGAGAGSGAGAGSGAGAGSGAGAGSGAGAGSGAGAGSGAGSGSGAGAGSGAGAGSGAGAGSGAGAGSGAGAGSGAGAGYGAGAGAGYGAGYGAGAGAGYGAGAGSGAGSGAGAGSGAGAGSGAGAGSGAGAGYGAGYGAGAGSGAASGAGAGAGAGAGTGSSGFGPYVAHGGYSGYEYAWSSESDFGTGSGAGAGSGAGAGAGAGAGSGAGAGYGAGVGAGYGAGYGAGAGAGYGAGAGSGTGSGAGAGSGAGAGYGAGVGAGYGAGAGSGAAFGAGAGAGAGSGAGAGSGAGAGSGAGAGSGAGAGSGAGAGYGAGYGAGVGAGYGAGAGSGAASGAGAGSGAGAGSGAGAGSGAGAGSGAGAGSGAGAGYGAGVGAGYGAGYGAGAGAGYGAGAGSGAASGAGAGSGAGAGAGSGAGAGSGAGAGSGAGAGSGAGSGAGAGSGAGAGSGAGAGYGAGAGSGAASGAGAGAGAGAGTGSSGFGPYVANGGYSGYEYAWSSESDFGTGSGAGAGSGAGAGSGAGAGSGAGAGSGAGAGYGAGVGAGYGAGYGAGAGAGYGAGAGSGAGSGAGAGSGAGAGSGAGAGSGAGAGSGAGAGSGAGAGSGAGAGYGAGAGSGAASGAGAGSGAGAGSGAGAGSGAGAGSGAGAGSGAGAGSGAGAGYGAGVGAGYGVGYGAGAGAGYGAGAGSGAGSGAGAGSGAGAGSGAGAGSGAGAGSGAGSGAGAGSGAGAGSGAGAGSGAGSGAGAGSGAGAGYGVGYGAGAGAGYGAGAGSGAGSGAGAGSGAGAGSGAGAGSGAGSGAGAGSGAGAGSGAGAGSGAGAGYGAGVGAGYGVGYGAGAGAGYGAGAGSGAGSGAGAGSGAGAGSGAGAGSGAGAGSGAGAGSGAGAGSGAGAGSGAGSGAGAGSGAGAGSGAGAGSGAGAGSGAGSGAGAGSGAGAGSGAGAGSGAGAGYGAGVGAGYGVGYGAGVGAGYGAGAGSGAASGAGAGSGAGAGAGSGAGAGSGAGAGSGAGAGSGAGAGSGAGAGSGAGAGYGAGYGAGVGAGYGAGAGVGYGAGAGAGYGAGAGSGAASGAGAGAGSGAGAGTGAGAGSGAGAGYGAGAGSGAASGAGAGAGAGAGTGSSGFGPYVANGGYSGYEYAWSSESDFGTGSGAGAGSGAGAGSGAGAGSGAGAGSGAGAGYGAGVGAGYGAGAGSGAGSGAGAGSGAGAGSGAGAGSGAGAGSGAGAGYGAGAGSGTGSGAGAGSGAGAGSGAGAGSGAGAGSGAGAGSGAGAGSGVGAGYGVGYGAGAGAGYGVGYGAGAGAGYGAGAGSGTGSGAGAGSGAGAGSGAGAGSGAGAGSGAGAGSGAGAGSGAGAGYGAGVGAGYGVGYGAGAGAGYGAGAGSGAGSGAGAGSGAGAGSGAGAGSGAGAGSGAGSGAGAGSGAGAGSGAGAGSGAGSGAGAGSGAGAGYGVGYGAGAGAGYGAGAGSGAGSGAGAGSGAGAGSGAGAGSGAGSGAGAGSGAGAGSGAGAGSGAGAGYGAGVGAGYGVGYGAGAGAGYGAGAGSGAGSGAGAGSGAGAGSGAGAGSGAGAGSGAGAGSGAGAGSGAGAGSGAGSGAGAGSGAGAGSGAGAGSGAGAGYGAGVGAGYGVGYGAGAGAGYGAGAGSGAASGAGAGAGAGAGTGSSGFGPYVANGGYSGYEYAWSSESDFGTGSGAGAGSGAGAGSGAGAGYGAGYGAGVGAGYGAGAGVGYGAGAGAGYGAGAGSGAASGAGAGAGAGAGSGAGAGSGAGAGAGSGAGAGYGAGYGIGVGAGYGAGAGVGYGAGAGAGYGAGAGSGAASGAGAGSGAGAGSGAGAGSGAGAGSGAGAGSGAGAGSGAGAGYGAGYGAGVGAGYGAGAGVGYGAGAGAGYGAGAGSGAASGAGAGAGAGAGAGSGAGAGSGAGAGSGAGAGSGAGAGSGAGAGSGAGAGSGAGAGSGAGAGSGAGAGYGAGVGAGYGAGYGGAGAGYGAGAGSGAASGAGAGSGAGAGSGAGAGSGAGAGSGAGAGSGAGAGYGAGAGSGAASGAGAGAGAGAGTGSSGFGPYVNGGYSGYEYAWSSESDFGTGSGAGAGSGAGAGSGAGAGYGAGVGAGYGAGYGAGAGAGYGAGAGSGAASGAGAGSGAGAGSGAGAGSGAGAGSGAGSGAGAGSGAGAGSGAGAGSGAGAGSGAGAGSGAGAGYGAGVGAGYGAGYGAGAGAGYGAGAGSGAASGAGAGSGAGAGAGSGAGAGSGAGAGSGAGAGSGAGAGSGAGAGSGAGSGAGAGSGAGAGYGAGYGAGVGAGYGAGAGVGYGAGAGAGYGAGAGSGAASGAGAGSGSGAGSGAGAGSGAGAGSGAGAGAGSGAGAGSGAGAGSGAGAGYGAGYGAGAGSGAASGAGAGAGAGAGTGSSGFGPYVANGGYSGYEYAWSSESDFGTGSGAGAGSGAGAGSGAGAGYGAGVGAGYGAGYGAGAGAGYGAGAGSGAGSGAGAGSGAGAGSGAGAGSGAGAGSGAGAGSGAGAGSGAGAGSGAGAGYGAGYGAGAGAGYGAGAGVGYGAGAGAGYGAGAGSGAGSGAGAGSGSGAGAGSGSGAGSGAGAGSGAGAGSGAGAGSGAGAGSGAGAGSGAGAGSGAGAGYGAGYGIGVGAGYGAGAGVGYGAGAGAGYGAGAGSGAASGAGAGSGAGAGSGAGAGSGAGAGSGAGAGSGAGAGSGAGAGSGAGAGSGAGAGSGAGAGYGAGAGVGYGAGAGSGAASGAGAGSGAGAGSGAGAGSGAGAGSGAGAGSGAGAGSGAGAGSGAGSGAGAGSGAGAGYGAGYGAGVGAGYGAGAGYGAGYGVGAGAGYGAGAGSGAGSGAGAGSGAGAGSGAGAGSGAGAGSGAGAGSGAGSGAGAGYGAGAGAGYGAGAGAGYGAGAGSGAASGAGAGAGAGSGAGAGSGAGAGSGAGSGAGAGSGAGAGYGAGAGSGAASGAGAGSGAGAGAGAGAGAGSGAGAGSGAGAGYGAGAGSGAASGAGAGAGAGTGSSGFGPYVANGGYSRREGYEYAWSSKSDFETGSGAASGAGAGAGSGAGAGSGAGAGSGAGAGSGAGAGGSVSYGAGRGYGQGAGSAASSVSSASSRSYDYSRRNVRKNCGIPRRQLVVKFRALPCVNC

SEQ ID NO: 8 - protein, 262 aa, Bombyx mori
MKPIFLVLLVATSAYAAPSVTINQYSDNEIPRDIDDGKASSVISRAWDYVDDTDKSIAILNVQEILKDMASQGDYASQASAVAQTAGIIAHLSAGIPGDACAAANVINSYTDGVRSGNFAGFRQSLGPFFGHVGQNLNLINQLVINPGQLRYSVGPALGCAGGGRIYDFEAAWDAILASSDSSFLNEEYCIVKRLYNSRNSQSNNIAAYITAHLLPPVAQVFHQSAGSITDLLRGVGNGNDATGLVANAQRYIAQAASQVHV

SEQ ID NO: 9 - protein, 1186 aa, Bombyx mori
MRFVLCCTLIALAALSVKAFGHHPGNRDTVEVKNRKYNAASSESSYLNKDNDSISAGAHRAKSVEQSQDKSKYTSGPEGVSYSGRSQNYKDSKQAYADYHSDPNGGSASAGQSRDSSLRERNVHYVSDGEAVAASSDARDENRSAQQNAQANWNADGSYGVSADRSGSASSRRRQANYYSDKDITAASKDDSRADSSRRSNAYYNRDSDGSESAGLSDRSASSSKNDNVFVYRTKDSIGGQAKSSRSSHSQESDAYYNSSPDGSYNAGTRDSSISNKKKASSTIYADKDQIRAANDRSSSKQLKQSSAQISSGPEGTSVSSKDRQYSNDKRSKSDAYVGRDGTVAYSNKDSEKTSRQSNTNYADQNSVRSDSAASDQTSKSYDRGYSDKNIVAHSSGSRGSQNQKSSSYRADKDGFSSSTNTEKSKFSSSNSVVETSDGASASRESSAEDTKSSNSNVQSDEKSASQSSSSRSSQESASYSSSSSSSTLSEDSSEVDIDLGNLGWWWNSDNKVQRAAGGATKSGASSSTQATTVSGADDSADSYTWWWNPRRSSSSSSSASSSSSGSNVGGSSQSSGSSTSGSNARGHLGTVSSTGSTSNTDSSSKSAGSRTSGGSSTYGYSSSHRGGSVSSTGSSSNTDSSTKNAGSSTSGGSSTYGYSSSHRGGSVSSTGSSSNTDSSTKSAGSSTSGGSSTYGYSSRHRGGRVSSTGSSSTTDASSNSVGSSTSGGSSTYGYSSNSRDGSVSSTGSSSNTDSNSNSAGSSTSGGSSTYGYSSNSRDGSVSSTGSSSNTDSNSNSAGSSTSGGSSTYGYSSNSRDGSVSSTGSSSNTDASTDLTGSSTSGGSSTYGYSSDSRDGSVSSTGSSSNTDASTDLAGSSTSGGSSTYGYSSDCGDGSVSSTGSSSNTDASTDLAGSSTSGGSSTYGYSSDSRDGSVSSTGSSSNTDASTDLAGSSTSGGSSTYGYSSNSRDGSVSSTGSSSNTDASTDLTGSSTSGGSSTYGYSSSNRDGSVLATGSSSNTDASTTEESTTSAGSSTEGYSSSSHDGSVTSTDGSSTSGGASSSSASTAKSDAASSEDGFWWWNRRKSGSGHKSATVQSSTTDKTSTDSASSTDSTSSTSGASTTTSGSSSTSGGSSTSDASSTSSSVSRSHHSGVNRLLHKPGQGKICLCFENIFDIPYHLRKNIGV

SEQ ID NO: 10 - protein, 900 aa, Bombyx mori
MKIPYVLLFLVGVAVVNALPNPLFGGLVKSLSKKKQIFEDKFENLKENVGEKFENLKENVGEKVENLKENVGEKLENIKEKAGEKFENLKDNVGEKFENLKDNVGDKLEAAKEKAGEIKKKLVDVGEDLKDELTEDKKIKISISKDEGLTLEKEGYKSDYDRNEYEERGSEHQEDNDSDGSYSKGSEYEKYGEEEKYEERRTHDKFSIGKNGISAERTKSKRGERKEVEGEYEKDYERKENNGGSSEYSERERESLEKSKERYGEQSSKSFSLGKSGLKKQDNSKSYSDKEESKLEKEKKYEKKTKINNERQLDEDENERRTVVGRDEQRQDDQSRDDQSRDDQSQDEETGSDDSDKNRGKDTDDKYSETGTNKSSETKTGKRDGSKSGVTVEREKSESNKKSREFENKEAESSTYRDKNRSVNSGSERKSSGKDEEYSEQNSSNKSFNDGDASADYQTKSKKVEKNSARDKKEKEKTDTRNSDGTYKTSEREKEQSSRVNQSKGSNSRDSSESDKSGRKVNKETETYSDKDAQTSESERTQSKDNGGLKEKSSQSKNYGRDEKYSEEKERSSTGKFGSNDSRARSTKAEEEHVRKSQEETHSEQREKTRSDGVTKYNDGDEHFDSDDTEKTKPNGRSPSHKDTEKAKPNDRSSSDKDTEKTFDKNIDNKRPKDGSSSDKNVEQERENYKSESSRNEFENQKSAHSRYEDNGGLKEKSSQSKNYGRDEKYSEEKERSSTGKSGSNDSRARSTKAEEEHVRKSQEETHSEQRGRTRSDGATTSNDNDKQYDSDDKNNSSTKHKKTVMRSEQSDSSQNENSTSESKKFAKTDGSNKYEAESSSHKQQEARKQSNRVVEKSTDGDNEESYRSESSSSSSSSSSSSRSSSSSTYTGSHDDSSEE

SEQ ID NO: 11 - protein, 1271 aa, Bombyx mori
MNCKVALFLIVAIVAVQALPCQESRPRRCGYRYGCGGGRGRGSGVRRLDSGADDNQGRSCLVGGSAESNDEDSDDRLSVINNTEGHATSSSFDEQSSSARQSSSSYQSQSYNKDSSSTNESSDGGSGSGRTGSAGENGENSDDSSGATKGNSSKSSSSSQGQSASSSSSDEKSSQSSSNSSNNSKSSSQSSSSQNSSGSKGSGSEESSNGGSGSGRTGSAGGTDEDSDDSSGATKGNSSKSSSSSQGQSASSSSSDENSSQSSSNSSNNSKSSSQSSSGQNSSGSKGSGSEESSNGGSGSGRNGSVGGTDEDSDDSSGATKGNSSKSSSSSQGQSASSSSSDEKSSQSSSNSSNNSKSSSQSSSGQNSSGSKGSGSEESSNGGSGSGRNGSAGGTDEDSDDSSGATKGNSSKSSSSSQGQSASSSSSDEKSSQSSSNSSNNSKSSSQSSSGQNSSGSKGSGSEESSNGGSGSGRNGSAGGTDEDSDDSSGATKGNSSKSSSSSQGQSASSSSSDEKSSQSSSNSSNNSKSSSQSSSGQNSSGSKGSGSEESSNGGSGSGRTGSAGETDEDSDDSSGATKGNSSKSSSSSQGKSASSSSSDEKSSQSSSNSSNNSKSSSQSSSSNNSSGSKGSGSEESSNGGSGSGRTGSAGGSDEDSDDSSGATKGNSSKSSSSSQGQSASSSSSDEKSSQSNSNSSNNSKSSSQSSSSNNSSGSKGSGSEESSNGGSGSGRTGSAGGTDEDSDDSSGATKGNSSKSSSSSQGKSASSSSSDEKSSQSSSNSSNNSKSSSQSSSSKNSSGSKGSGSEESSNGGSGSGRTGSAGGTDEDSDDSSGATKGNSSKSSSSSQGKSASSSSSDEKSSQSNSNSSNNSKSSSQSSSSKNSSGSKGSGSEESSNGGSGSGRTGSAGGTDEDSDDSSGATKGNSSKSSSSSQGKSASSSSSNEKSSQSSSNSSNNSKSSSQSSSSKNSSGSKGSGSSESGDKKSSSRGSSGDNSDDDQTDSARSNSKRSTSSDASTKKSSSRKSSNHRSSRSQQAHSSSSKQAQSSSSQQAQNSRSQQAHSSRSQQAHSSSSKQAQSSSSKQAQSSSSKQAQSSSSKQAQSSSSQQAQSSRSQQAHSSRSQQAHSSSSKQAQSSSSKQAQSSSSKQAQSSSSKQAQSSSSQQAQSSRSQQAHSSRSETDSKSSNSGGHSNHSSRTEQKSSAKAISSSEQSQNFSSSSQKSAEAADGSESTQSASEYSSSQSKASSSFSASSASESSSLSSDVNFEEKTD

SEQ ID NO: 12 - protein, 748 aa, Nephila clavipes
QGAGAAAAAAGGAGQGGYGGLGGQGAGQGGYGGLGGQGAGQGAGAAAAAAAGGAGQGGYGGLGSQGAGRGGQGAGAAAAAAGGAGQGGYGGLGSQGAGRGGLGGQGAGAAAAAAAGGAGQGGYGGLGNQGAGRGGQGAAAAAAGGAGQGGYGGLGSQGAGRGGLGGQGAGAAAAAAGGAGQGGYGGLGGQGAGQGGYGGLGSQGAGRGGLGGQGAGAAAAAAAGGAGQGGLGGQGAGQGAGASAAAAGGAGQGGYGGLGSQGAGRGGEGAGAAAAAAGGAGQGGYGGLGGQGAGQGGYGGLGSQGAGRGGLGGQGAGAAAAGGAGQGGLGGQGAGQGAGAAAAAAGGAGQGGYGGLGSQGAGRGGLGGQGAGAVAAAAAGGAGQGGYGGLGSQGAGRGGQGAGAAAAAAGGAGQRGYGGLGNQGAGRGGLGGQGAGAAAAAAAGGAGQGGYGGLGNQGAGRGGQGAAAAAGGAGQGGYGGLGSQGAGRGGQGAGAAAAAAVGAGQEGIRGQGAGQGGYGGLGSQGSGRGGLGGQGAGAAAAAAGGAGQGGLGGQGAGQGAGAAAAAAGGVRQGGYGGLGSQGAGRGGQGAGAAAAAAGGAGQGGYGGLGGQGVGRGGLGGQGAGAAAAGGAGQGGYGGVGSGASAASAAASRLSSPQASSRVSSAVSNLVASGPTNSAALSSTISNVVSQIGASNPGLSGCDVLIQALLEVVSALIQILGSSSIGQVNYGSAGQATQIVGQSVYQALG

SEQ ID NO: 13 - protein, 627 aa, Nephila clavipes
PGGYGPGQQGPGGYGPGQQGPSGPGSAAAAAAAAAAGPGGYGPGQQGPGGYGPGQQGPGRYGPGQQGPSGPGSAAAAAAGSGQQGPGGYGPRQQGPGGYGQGQQGPSGPGSAAAASAAASAESGQQGPGGYGPGQQGPGGYGPGQQGPGGYGPGQQGPSGPGSAAAAAAAASGPGQQGPGGYGPGQQGPGGYGPGQQGPSGPGSAAAAAAAASGPGQQGPGGYGPGQQGPGGYGPGQQGLSGPGSAAAAAAAGPGQQGPGGYGPGQQGPSGPGSAAAAAAAAAGPGGYGPGQQGPGGYGPGQQGPSGAGSAAAAAAAGPGQQGLGGYGPGQQGPGGYGPGQQGPGGYGPGSASAAAAAAGPGQQGPGGYGPGQQGPSGPGSASAAAAAAAAGPGGYGPGQQGPGGYAPGQQGPSGPGSASAAAAAAAAGPGGYGPGQQGPGGYAPGQQGPSGPGSAAAAAAAAAGPGGYGPAQQGPSGPGIAASAASAGPGGYGPAQQGPAGYGPGSAVAASAGAGSAGYGPGSQASAAASRLASPDSGARVASAVSNLVSSGPTSSAALSSVISNAVSQIGASNPGLSGCDVLIQALLEIVSACVTILSSSSIGQVNYGAASQFAQVVGQSVLSAF